European Patent Application EP 4 265 631 A2, published October 25, 2023. Title: LIVE-ATTENUATED FLAVIRUSES WITH HETEROLOGOUS ANTIGENS. Applicant: Katholieke Universiteit Leuven. Application EP. The sequence listing filed with the application follows.

SEQUENCE LISTING (48 sequences)

SEQ ID NO: 1 - DNA, 1744 bp, synthetic construct
  misc_feature 1..1744: note = 5' end of YFV with heterologous antigen
  source 1..1744: mol_type = other DNA
agtaaatcctgtgtgctaattgaggtgcattggtctgcaaatcgagttgctaggcaataaacacatttggattaattttaatcgttcgttgagcgattagcagagaactgaccagaacatgtctggtcgtaaagctcagggaaaaaccctgggcgtcaatatggtacgacgaggagttcgcggatccgtttaaacctcgtccccgccgggtcacccggccagcgacatggaggcccagaataccctccttgacagtcttgacgtgcgcagctcaggggcatgatgtgactgtcgcccgtacatttagcccatacatccccatgtataatcatttgcatccatacattttgatggccgcacggcgcgaagcaaaaattacggctcctcgctgcagacctgcgagcagggaaacgctcccctcacagacgcgttgaattgtccccacgccgcgcccctgtagagaaatataaaaggttaggatttgccactgaggttcttctttcatatacttccttttaaaatcttgctaggatacagttctcacatcacatccgaacataaacaaccatgacagtcaacactaagacctatagtgagagagcagaaactcatgcctcaccagtagcacaacgattatttcgattaatggaactgaagaaaaccaatttatgtgcatcaattgatgttgataccactaaggaattccttgaattaattgataaattgggtccttatgtatgcttaatcaagactcatattgatataatcaatgatttttcctatgaatccactattgaaccattattagaactttcacgtaaacatcaatttatgatttttgaagatagaaaatttgctgatattggtaataccgtgaagaaacaatatattggtggagtttataaaattagtagttgggcagatattactaatgctcatggtgtcactgggaatggagtagttgaaggattaaaacagggagctaaagaaaccaccaccaaccaagagccaagagggttattgatgttagctgaattatcatcagtgggatcattagcatatggagaatattctcaaaaaactgttgaaattgctaaatccgataaggaatttgttattggatttattgcccaacgtgatatgggtggacaagaagaaggatttgattggcttattatgacacctggagttggattagatgataaaggtgatggattaggacaacaatatagaactgttgatgaagttgttagcactggaactgatattatcattgttggtagaggattgtttggtaaaggaagagatccagatattgaaggtaaaaggtatagagatgctggttggaatgcttatttgaaaaagactggccaattataatcagtactgacaataaaaagattcttgttttcaagaacttgtcatttgtatagtttttttatattgtagttgttctattttaatcaaatgttagcgtgatttatattttttttcgcctcgacatcatctgcccagatgcgaagttaagtgcgcagaaagtaatatcatgcgtcaatcgtatgtgaatgctggtcgctatactgtttaaacgagggacgcgggtccctgctgacctgtggcgacgtggaggagaaccccggtcctagcggccgcaaagcccagggtaagacactgggcgtgaacatggttcgtcgcggcgtccggtccttgtcaaacaaaataaaacaaaaaacaaaacaaattg

SEQ ID NO: 2 - protein, 21 aa, synthetic construct
  REGION 1..21: note = N terminal part of capsid
MSGRKAQGKTLGVNMVRRGVR

SEQ ID NO: 3 - protein, 270 aa, synthetic construct
  REGION 1..270: note = Hepatitis antigen
MTVNTKTYSERAETHASPVAQRLFRLMELKKTNLCASIDVDTTKEFLELIDKLGPYVCLIKTHIDIINDFSYESTIEPLLELSRKHQFMIFEDRKFADIGNTVKKQYIGGVYKISSWADITNAHGVTGNGVVEGLKQGAKETTTNQEPRGLLMLAELSSVGSLAYGEYSQKTVEIAKSDKEFVIGFIAQRDMGGQEEGFDWLIMTPGVGLDDKGDGLGQQYRTVDEVVSTGTDIIIVGRGLFGKGRDPDIEGKRYRDAGWNAYLKKTGQL

SEQ ID NO: 4 - protein, 51 aa, synthetic construct
  REGION 1..51: note = 2A peptide + N terminal part of capsid protein
EGRGSLLTCGDVEENPGPSGRKAQGKTLGVNMVRRGVRSLSNKIKQKTKQI

SEQ ID NO: 5 - DNA, 806 bp, synthetic construct
  misc_feature 1..806: note = YF17D based constructs with hepatitis antigen
  source 1..806: mol_type = other DNA
agtaaatcctgtgtgctaattgaggtgcattggtctgcaaatcgagttgctaggcaataaacacatttggattaattttaatcgttcgttgagcgattagcagagaactgaccagaacatgtctggtcgtaaagctcagggaaaaaccctgggcgtcaatatggtacgacgaggagttcgcggatccatggacatcgacccttataaagaatttggagctactgtggagttactctcgtttttgccttctgacttctttccttcagtacgagatcttctagataccgcctcagctctgtatcgggaagccttagagtctcctgagcattgttcacctcaccatactgcactcaggcaagcaattctttgctggggggaactaatgactctagctacctgggtgggtgttaatttggaagatccagcgtctagagacctagtagtcagttatgtcaacactaatatgggcctaaagttcaggcaactcttgtggtttcacatttcttgtctcacttttggaagagaaacagttatagagtatttggtgtctttcggagtgtggattcgcactcctccagcttatagaccaccaaatgcccctatcctatcaacacttccggagactactgttgttagacgacgaggcaggtccgagggacgcgggtccctgctgacctgtggcgacgtggaggagaaccccggtcctagcggccgcaaagcccagggtaagacactgggcgtgaacatggttcgtcgcggcgtccggtccttgtcaaacaaaataaaacaaaaaacaaaacaaattg

SEQ ID NO: 6 - protein, 229 aa, synthetic construct
  REGION 1..229: note = YFV based construct with hepatitis antigen
MSGRKAQGKTLGVNMVRRGVRGSMDIDPYKEFGATVELLSFLPSDFFPSVRDLLDTASALYREALESPEHCSPHHTALRQAILCWGELMTLATWVGVNLEDPASRDLVVSYVNTNMGLKFRQLLWFHISCLTFGRETVIEYLVSFGVWIRTPPAYRPPNAPILSTLPETTVVRRRGRSEGRGSLLTCGDVEENPGPSGRKAQGKTLGVNMVRRGVRSLSNKIKQKTKQI

SEQ ID NO: 7 - protein, 154 aa, synthetic construct
  REGION 1..154: note = Hepatis B antigen sequence
MDIDPYKEFGASVELLSFLPSDFFPSIRDLLDTASALYREALESPEHCSPHHTALRQAILCWGELMNLATWVGGNLEDPASREAVVSYVNVNMGLKIRQLLWFHISCLTFGRETVLEYLVSFGVWIRTPPAYRPQNAPILSTLPETTVVRRRGR

SEQ ID NO: 8 - DNA, 1429 bp, synthetic construct
  misc_feature 1..1429: note = YFV based construct with ovalbumin
  source 1..1429: mol_type = other DNA
agtaaatcctgtgtgctaattgaggtgcattggtctgcaaatcgagttgctaggcaataaacacatttggattaattttaatcgttcgttgagcgattagcagagaactgaccagaacatgtctggtcgtaaagctcagggaaaaaccctgggcgtcaatatggtacgacgaggagttcgcggatccatgggtagtatcggggcagcctccatggagttctgctttgacgtattcaaagagctcaaggttcatcatgctaacgaaaacattttttattgccccatcgccataatgagtgctctggccatggtgtatcttggggccaaagattcaacacggacacagataaacaaagtagtccgcttcgacaaattgcctggatttggcgattctatcgaagctcagtgcgggacatccgtgaatgtgcatagtagtctcagggatatcctcaaccagataacaaaaccaaatgacgtttattcttttagcctcgccagtcgcctttatgccgaggaacggtatcccattttgccagagtacttgcaatgtgtaaaagagttgtaccgaggcgggctcgaacccattaatttccagacagcagcagaccaagcaagagagcttataaatagctgggtagaatctcaaactaacggaattataagaaacgtgctccaaccaagttcagtggattctcagacagccatggtccttgttaatgccattgttttcaaaggtctttgggagaaagcatttaaagatgaggatacccaggctatgccctttcgagtaaccgaacaagagagtaagcccgtacaaatgatgtaccagataggattgtttagagtcgcctccatggctagtgagaagatgaagattctggagctcccctttgccagcggtacaatgagcatgcttgtcctgctccctgacgaggtgtcagggctcgaacaattggagagcattatcaacttcgagaaactcacagaatggactagtagcaatgtgatggaggaaaggaagattaaggtatatcttccacggatgaaaatggaagagaaatacaatctcacaagcgtactcatggctatgggaataacagatgtgttttcatccagcgccaacttgagcggcattagctctgccgaaagtctgaagatttcacaggccgtacatgccgcccacgctgaaataaatgaggctggcagggaagtagttgggagtgcagaggctggcgtagatgctgccagcgtatccgaggagttccgagccgatcacccttttctcttttgtatcaaacatattgctactaatgcagtcctctttttcggtcggtgtgtgagcccagagggacgcgggtccctgctgacctgtggcgacgtggaggagaaccccggtcctacaaaataaaacaaaaaacaaaacaaattg

SEQ ID NO: 9 - protein, 460 aa, synthetic construct
  REGION 1..460: note = YFV based construct with ovalbumin
MSGRKAQGKTLGVNMVRRGVRGSMGSIGAASMEFCFDVFKELKVHHANENIFYCPIAIMSALAMVYLGAKDSTRTQINKVVRFDKLPGFGDSIEAQCGTSVNVHSSLRDILNQITKPNDVYSFSLASRLYAEERYPILPEYLQCVKELYRGGLEPINFQTAADQARELINSWVESQTNGIIRNVLQPSSVDSQTAMVLVNAIVFKGLWEKAFKDEDTQAMPFRVTEQESKPVQMMYQIGLFRVASMASEKMKILELPFASGTMSMLVLLPDEVSGLEQLESIINFEKLTEWTSSNVMEERKIKVYLPRMKMEEKYNLTSVLMAMGITDVFSSSANLSGISSAESLKISQAVHAAHAEINEAGREVVGSAEAGVDAASVSEEFRADHPFLFCIKHIATNAVLFFGRCVSPEGRGSLLTCGDVEENPGPSGRKAQGKTLGVNMVRRGVRSLSNKIKQKTKQI

SEQ ID NO: 10 - protein, 386 aa, Gallus gallus
MGSIGAASMEFCFDVFKELKVHHANENIFYCPIAIMSALAMVYLGAKDSTRTQINKVVRFDKLPGFGDSIEAQCGTSVNVHSSLRDILNQITKPNDVYSFSLASRLYAEERYPILPEYLQCVKELYRGGLEPINFQTAADQARELINSWVESQTNGIIRNVLQPSSVDSQTAMVLVNAIVFKGLWEKAFKDEDTQAMPFRVTEQESKPVQMMYQIGLFRVASMASEKMKILELPFASGTMSMLVLLPDEVSGLEQLESIINFEKLTEWTSSNVMEERKIKVYLPRMKMEEKYNLTSVLMAMGITDVFSSSANLSGISSAESLKISQAVHAAHAEINEAGREVVGSAEAGVDAASVSEEFRADHPFLFCIKHIATNAVLFFGRCVSP

SEQ ID NO: 11 - DNA, 1064 bp, synthetic construct
  misc_feature 1..1064: note = YFV based constuct with EBNA 1 antigen
  source 1..1064: mol_type = other DNA
agtaaatcctgtgtgctaattgaggtgcattggtctgcaaatcgagttgctaggcaataaacacatttggattaattttaatcgttcgttgagcgattagcagagaactgaccagaacatgtctggtcgtaaagctcagggaaaaaccctgggcgtcaatatggtacgacgaggagttcgcggatccggtagaaggccatttttccaccctgtaggggaagccgattattttgaataccaccaagaaggtggcccagatggtgagcctgacgtgcccccgggagcgatagagcagggccccgcagatgacccaggagaaggcccaagcactggaccccggggtcagggtgatggaggcaggcgcaaaaaaggagggtggtttggaaagcatcgtggtcaaggaggttccaacccgaaatttgagaacattgcagaaggtttaagagctctcctggctaggagtcacgtagaaaggactaccgacgaaggaacttgggtcgccggtgtgttcgtatatggaggtagtaagacctccctttacaacctaaggcgaggaactgcccttgctattccacaatgtcgtcttacaccattgagtcgtctcccctttggaatggcccctggacccggcccacaacctggcccgctaagggagtccattgtctgttatttcatggtctttttacaaactcatatatttgctgaggttttgaaggatgcgattaaggaccttgttatgacaaagcccgctcctacctgcaatatcagggtgactgtgtgcagctttgacgatggagtagatttgcctccctggtttccacctatggtggaaggggctgccgcggagggtgatgacggagatgacggagatgaaggaggtgatggagatgagggtgaggaagggcaggaggagggacgcgggtccctgctgacctgtggcgacgtggaggagaaccccggtcctagcggccgcaaagcccagggtaagacactgggcgtgaacatggttcgtcgcggcgtccggtccttgtcaaacaaaataaaacaaaaaacaaaacaaattg

SEQ ID NO: 12 - protein, 315 aa, synthetic construct
  REGION 1..315: note = YVF based construct with EBNA1 antigen
MSGRKAQGKTLGVNMVRRGVRGSGRRPFFHPVGEADYFEYHQEGGPDGEPDVPPGAIEQGPADDPGEGPSTGPRGQGDGGRRKKGGWFGKHRGQGGSNPKFENIAEGLRALLARSHVERTTDEGTWVAGVFVYGGSKTSLYNLRRGTALAIPQCRLTPLSRLPFGMAPGPGPQPGPLRESIVCYFMVFLQTHIFAEVLKDAIKDLVMTKPAPTCNIRVTVCSFDDGVDLPPWFPPMVEGAAAEGDDGDDGDEGGDGDEGEEGQEEGRGSLLTCGDVEENPGPSGRKAQGKTLGVNMVRRGVRSLSNKIKQKTKQI

SEQ ID NO: 13 - protein, 238 aa, synthetic construct
  REGION 1..238: note = EBNA1 antigen
PFFHPVGEADYFEYLQEGGPDGEPDVPPGAIEQGPADDPGEGPSTGPRGQGDGGRRKKGGWFGKHRGQGGSNPKFENIAEGLRVLLARSHVERTTEEGTWVAGVFVYGGSKTSLYNLRRGTALAIPQCRLTPLSRLPFGMAPGPGPQPGPLRESIVCYFMVFLQTHIFAEVLKDAIKDLVMTKPAPTCNIKVTVCSFDDGVDLPPWFPPMVEGAAAEGDDGDDGDEGGDGDEGEEGQE

SEQ ID NO: 14 - DNA, 63 bp, synthetic construct
  misc_feature 1..63: note = cDNA for YFV capsid nterminal fragment
  source 1..63: mol_type = other DNA
atgtctggtcgtaaagctcagggaaaaaccctgggcgtcaatatggtacgacgaggagttcgc

SEQ ID NO: 15 - DNA, 60 bp, synthetic construct
  misc_feature 1..60: note = cDNA for capsid nterminal fragment
  source 1..60: mol_type = other DNA
agcggccgcaaagcccagggtaagacactgggcgtgaacatggttcgtcgcggcgtccgg

SEQ ID NO: 16 - protein, 18 aa, Thosea asigna
EGRGSLLTCGDVEENPGP

SEQ ID NO: 17 - protein, 12 aa, synthetic construct
  REGION 1..12: note = viral 2A cleaving peptide
  REGION 2..4: note = misc_feature - Xaa can be any naturally occurring amino acid
  SITE 9: note = misc_feature - Xaa can be any naturally occurring amino acid
LXXXGDVEXPGP

SEQ ID NO: 18 - protein, 13 aa, Thosea asigna
LLTCGDVEENPGP

SEQ ID NO: 19 - DNA, 56 bp, synthetic construct
  misc_feature 1..56: note = pcr primer
  source 1..56: mol_type = other DNA
aagctcagggaaaaaccctgggcgtcaatatggtacgacgaggagttcgcggatcc

SEQ ID NO: 20 - DNA, 60 bp, synthetic construct
  misc_feature 1..60: note = pcr primer
  source 1..60: mol_type = other DNA
gtgtcttaccctgggctttgcggccgctaggaccggggttctcctccacgtcgccacagg

SEQ ID NO: 21 - DNA, 60 bp, synthetic construct
  misc_feature 1..60: note = pcr primer
  source 1..60: mol_type = other DNA
gtcaatatggtacgacgaggagttcgcggatccgtttaaacctcgtccccgccgggtcac

SEQ ID NO: 22 - DNA, 60 bp, synthetic construct
  misc_feature 1..60: note = pcr primer
  source 1..60: mol_type = other DNA
gtcgccacaggtcagcagggacccgcgtccctcgtttaaacagtatagcgaccagcattc

SEQ ID NO: 23 - DNA, 60 bp, synthetic construct
  misc_feature 1..60: note = pcr primer
  source 1..60: mol_type = other DNA
cagaacatgtctggtcgtaaagctcagggaaaaaccctgggcgtcaatatggtacgacga

SEQ ID NO: 24 - DNA, 60 bp, synthetic construct
  misc_feature 1..60: note = pcr primer
  source 1..60: mol_type = other DNA
accctgggctttgcggccgctaggaccggggttctcctccacgtcgccacaggtcagcag

SEQ ID NO: 25 - DNA, 60 bp, synthetic construct
  misc_feature 1..60: note = pcr primer
  source 1..60: mol_type = other DNA
ccggacgccgcgacgaaccatgttcacgcccagtgtcttaccctgggctttgcggccgct

SEQ ID NO: 26 - DNA, 60 bp, synthetic construct
  misc_feature 1..60: note = pcr primer
  source 1..60: mol_type = other DNA
cctgggcgtcaatatggtacgacgaggagttcgcggatccatggacatcgacccttataa

SEQ ID NO: 27 - DNA, 60 bp, synthetic construct
  misc_feature 1..60: note = pcr primer
  source 1..60: mol_type = other DNA
cctccacgtcgccacaggtcagcagggacccgcgtccctccgcgagggcctttccctcgg

SEQ ID NO: 28 - DNA, 60 bp, synthetic construct
  misc_feature 1..60: note = pcr primer
  source 1..60: mol_type = other DNA
gtcttaccctgggctttgcggccgctaggaccggggttctcctccacgtcgccacaggtc

SEQ ID NO: 29 - DNA, 60 bp, synthetic construct
  misc_feature 1..60: note = pcr primer
  source 1..60: mol_type = other DNA
tggaggagaaccccggtcctagcggccgcaaagcccagggtaagacactgggcgtgaaca

SEQ ID NO: 30 - DNA, 60 bp, synthetic construct
  misc_feature 1..60: note = pcr primer
  source 1..60: mol_type = other DNA
taagacactgggcgtgaacatggttcgtcgcggcgtccggtccttgtcaaacaaaataaa

SEQ ID NO: 31 - DNA, 60 bp, synthetic construct
  misc_feature 1..60: note = pcr primer
  source 1..60: mol_type = other DNA
tgacgcccagggtttttccctgagctttacgaccagacatgttctggtcagttctctgct

SEQ ID NO: 32 - DNA, 60 bp, synthetic construct
  misc_feature 1..60: note = pcr primer
  source 1..60: mol_type = other DNA
tcgatgtccatggatccgcgaactcctcgtcgtaccatattgacgcccagggtttttccc

SEQ ID NO: 33 - DNA, 57 bp, synthetic construct
  misc_feature 1..57: note = pcr primer
  source 1..57: mol_type = other DNA
tggattaattttaatcgttcgttgagcgattagcagagaactgaccagaacatgtct

SEQ ID NO: 34 - DNA, 57 bp, synthetic construct
  misc_feature 1..57: note = pcr primer
  source 1..57: mol_type = other DNA
cctccacgtcgccacaggtcagcagggacccgcgtccctcggacctgcctcgtcgtc

SEQ ID NO: 35 - DNA, 60 bp, synthetic construct
  misc_feature 1..60: note = pcr primer
  source 1..60: mol_type = other DNA
tgtttccaatttgttttgttttttgttttattttgtttgacaaggaccggacgccgcgac

SEQ ID NO: 36 - DNA, 60 bp, synthetic construct
  misc_feature 1..60: note = pcr primer
  source 1..60: mol_type = other DNA
gggcgtcaatatggtacgacgaggagttcgcggatccatgggtagaaggccatttttcca

SEQ ID NO: 37 - DNA, 60 bp, synthetic construct
  misc_feature 1..60: note = pcr primer
  source 1..60: mol_type = other DNA
cctccacgtcgccacaggtcagcagggacccgcgtccctcctcctgcccttcctcaccct

SEQ ID NO: 38 - protein, 24 aa, Foot-and-mouth disease virus
APVKQTLNFDLLKLAGDVESNPGP

SEQ ID NO: 39 - protein, 19 aa, Porcine teschovirus-1
ATNFSLLKQAGDVEENPGP

SEQ ID NO: 40 - protein, 20 aa, Equine rhinitis A virus
QCTNYALLKLAGDVESNPGP

SEQ ID NO: 41 - protein, 29 aa, synthetic construct
  REGION 1..29: note = Yellow fever capsid fragment + Hbc fragment
MSGRKAQGKTLGVNMVRRGVRGSMDIDPY

SEQ ID NO: 42 - protein, 30 aa, synthetic construct
  REGION 1..30: note = Hbc fragment - T2A peptide - Yeloow fever fragment
RRRGRSEGRGSLLTCGDVEENPGPSGRKAQ

SEQ ID NO: 43 - DNA, 63 bp, Yellow fever virus; identical to SEQ ID NO: 14
  source 1..63: mol_type = genomic DNA

SEQ ID NO: 44 - DNA, 58 bp, synthetic construct
  misc_feature 1..58: note = codon modified YFV capsid
  source 1..58: mol_type = other DNA
cggccgcaaagcccagggtaagacactgggcgtgaacatggttcgtcgcggcgtccgg

SEQ ID NO: 45 - protein, 21 aa, Yellow fever virus
MSGRKAQGKTLGVNMVRRGVR

SEQ ID NO: 46 - protein, 8 aa, synthetic construct
  REGION 1..8: note = 2A peptide consensus sequence
  SITE 2: note = misc_feature - Xaa can be any naturally occurring amino acid
  SITE 4: note = misc_feature - Xaa can be any naturally occurring amino acid
DXEXNPGP

SEQ ID NO: 47 - protein, 4 aa, synthetic construct
  REGION 1..4: note = 2A cleavage site
NPGP

SEQ ID NO: 48 - protein, 5 aa, synthetic construct
  REGION 1..5: note = 2A cleavage site
NPGPS